European Patent Specification EP 3 794 012 B1, published October 18, 2023. Title: COMPOSITIONS AND METHODS FOR CHEMICAL CLEAVAGE AND DEPROTECTION OF SURFACE-BOUND OLIGONUCLEOTIDES. Applicant: Illumina, Inc.; Illumina Cambridge Limited. The sequence listing filed with the application follows.

SEQUENCE LISTING (8 sequences)

SEQ ID NO: 1 - DNA, 29 bp, Artificial Sequence
  Synthetic; P5:  paired end
  misc_feature (23)..(23): n = u
aatgatacggcgaccaccgaganctacac

SEQ ID NO: 2 - DNA, 24 bp, Artificial Sequence
  Synthetic; P7:  paired end
  misc_feature (22)..(22): n = 8-oxo-guanine
caagcagaagacggcatacganat

SEQ ID NO: 3 - DNA, 39 bp, Artificial Sequence
  Synthetic; P5 primer with poly-T spacer
  misc_feature (1)..(1): 5'-alkyne
  misc_feature (33)..(33): n = u
ttttttttttaatgatacggcgaccaccgaganctacac

SEQ ID NO: 4 - DNA, 34 bp, Artificial Sequence
  Synthetic; P7 primer with poly-T spacer
  misc_feature (1)..(1): 5'-alkyne
  misc_feature (32)..(32): n = 8-oxo-guanine
ttttttttttcaagcagaagacggcatacganat

SEQ ID NO: 5 - DNA, 35 bp, Artificial Sequence
  Synthetic; P15 primer
  misc_feature (1)..(1): 5'-alkyne
  misc_feature (29)..(29): n = allyl t nucleoside
ttttttaatgatacggcgaccaccgaganctacac

SEQ ID NO: 6 - DNA, 33 bp, Artificial Sequence
  Synthetic; P17 primer
  misc_feature (1)..(1): 5'-alkyne
  misc_feature (7)..(7): diol linker
  misc_feature (8)..(8): diol linker
  misc_feature (9)..(9): diol linker
ttttttnnncaagcagaagacggcatacgagat

SEQ ID NO: 7 - DNA, 20 bp, Artificial Sequence
  Synthetic; P5: single read
aatgatacggcgaccaccga

SEQ ID NO: 8 - DNA, 21 bp, Artificial Sequence
  Synthetic; P7: single read
caagcagaagacggcatacga